European Patent Application EP 4 538 379 A1, published April 16, 2025. Title: METHOD FOR MAKING CELLS, METHOD FOR PRODUCING HETEROMULTIMERIC PROTEIN, METHOD FOR PRODUCING BISPECIFIC ANTIBODY, VECTOR SET, MAMMALIAN CELLS, CHO CELLS, AND METHOD FOR MAKING CELL POOL. Applicant: FUJIFILM Corporation. The sequence listing filed with the application follows.

SEQUENCE LISTING (4 sequences)

SEQ ID NO: 1 - protein, 26 aa, Homo sapiens
  REGION 1..26: note = Fibronectin secretion leader
MLRGPGPGLLLLAVQCLGTAVPSTGA

SEQ ID NO: 2 - protein, 25 aa, Cricetulus griseus
  REGION 1..25: note = Fibronectin secretion leader
MLRGPGPGLLLAVLCLGTAVRCTEA

SEQ ID NO: 3 - DNA, 78 bp, Homo sapiens
  misc_feature 1..78: note = Fibronectin secretion leader
  source 1..78: mol_type = genomic DNA
atgctgagaggccctggacctggactgctgctgctggctgtgcagtgtctgggaaccgccgtgccttctaccggcgcc

SEQ ID NO: 4 - DNA, 75 bp, Cricetulus griseus
  misc_feature 1..75: note = Fibronectin secretion leader
  source 1..75: mol_type = genomic DNA
atgctcaggggtccgggacccgggctgctgctggccgtcctgtgcctggggacagcggtgcgctgtaccgaagcc